European Patent Application EP 4 775 680 A1, published July 15, 2026. Title: タンパク質又はペプチドの製造方法、5´キャップ化ポリヌクレオチドの製造方法、及びそれらの製造方法に用いるための試薬. Applicant: 国立大学法人東海国立大学機構. The sequence listing filed with the application follows.

SEQUENCE LISTING (71 sequences)

SEQ ID NO: 1 - protein, 883 aa, T7 phage
MNTINIAKNDFSDIELAAIPFNTLADHYGERLAREQLALEHESYEMGEARFRKMFERQLKAGEVADNAAAKPLITTLLPKMIARINDWFEEVKAKRGKRPTAFQFLQEIKPEAVAYITIKTTLACLTSADNTTVQAVASAIGRAIEDEARFGRIRDLEAKHFKKNVEEQLNKRVGHVYKKAFMQVVEADMLSKGLLGGEAWSSWHKEDSIHVGVRCIEMLIESTGMVSLHRQNAGVVGQDSETIELAPEYAEAIATRAGALAGISPMFQPCVVPPKPWTGITGGGYWANGRRPLALVRTHSKKALMRYEDVYMPEVYKAINIAQNTAWKINKKVLAVANVITKWKHCPVEDIPAIEREELPMKPEDIDMNPEALTAWKRAAAAVYRKDRARKSRRISLEFMLEQANKFANHKAIWFPYNMDWRGRVYAVSMFNPQGNDMTKGLLTLAKGKPIGKEGYYWLKIHGANCAGVDKVPFPERIKFIEENHENIMACAKSPLENTWWAEQDSPFCFLAFCFEYAGVQHHGLSYNCSLPLAFDGSCSGIQHFSAMLRDEVGGRAVNLLPSETVQDIYGIVAKKVNEILQADAINGTDNEVVTVTDENTGEISEKVKLGTKALAGQWLAHGVTRSVTKRSVMTLAYGSKEFGFRQQVLEDTIQPAIDSGKGPMFTQPNQAAGYMAKLIWESVSVTVVAAVEAMNWLKSAAKLLAAEVKDKKTGEILRKRCAVHWVTPDGFPVWQEYKKPIQTRLNLMFLGQFRLQPTINTNKDSEIDAHKQESGIAPNFVHSQDGSHLRKTVVWAHEKYGIESFALIHDSFGTIPADAANLFKAVRETMVDTYESCDVLADFYDQFADQLHESQLDKMPALPAKGNLNLRDILESDFAFA

SEQ ID NO: 2 - RNA, 264 nt, synthetic construct
  source 1..264: mol_type = other RNA
gggagccaccatggactacaaggacgacgacgacaagatcatcgactataaagacgacgacgataaaggtggcgactataaggacgacgacgacaaagccatcaacagcgacagcgagtgccccctgagccacgacggctactgcctgcacgacggcgtgtgcatgtacatcgaggccctggacaagtacgcctgcaactgcgtggtgggctacatcggcgagagatgccagtacagagacctgaagtggtgggagctgagact

SEQ ID NO: 3 - RNA, 26 nt, synthetic construct
  source 1..26: mol_type = other RNA
gccacctctctgtactggcatctctc

SEQ ID NO: 4 - RNA, 50 nt, synthetic construct
  source 1..50: mol_type = other RNA
gacagtctgctcgaagcggccgctctagaatctctgtactggcatctctc

SEQ ID NO: 5 - RNA, 50 nt, synthetic construct
  source 1..50: mol_type = other RNA
gacagtctgctcgaagcggccgctctagaaccgcgtataattccactgcg

SEQ ID NO: 6 - RNA, 620 nt, synthetic construct
  source 1..620: mol_type = other RNA
ggcgcatattaaggtgacgcgtgtggcctcgaacaccgagcgaccctgcagcgacccgcttaaaagcttggcaatccggtactgttggtaaagccaccatggtcttcacactcgaagatttcgttggggactggcgacagacagccggctacaacctggaccaagtccttgaacagggaggtgtgtccagtttgtttcagaatctcggggtgtccgtaactccgatccaaaggattgtcctgagcggtgaaaatgggctgaagatcgacatccatgtcatcatcccgtatgaaggtctgagcggcgaccaaatgggccagatcgaaaaaatttttaaggtggtgtaccctgtggatgatcatcactttaaggtgatcctgcactatggcacactggtaatcgacggggttacgccgaacatgatcgactatttcggacggccgtatgaaggcatcgccgtgttcgacggcaaaaagatcactgtaacagggaccctgtggaacggcaacaaaattatcgacgagcgcctgatcaaccccgacggctccctgctgttccgagtaaccatcaacggagtgaccggctggcggctgtgcgaacgcattctggcgtaattctag

SEQ ID NO: 7 - DNA, 20 bp, synthetic construct
  source 1..20: mol_type = other DNA
aatatgcgccctagaattac

SEQ ID NO: 8 - RNA, 22 nt, synthetic construct
  source 1..22: mol_type = other RNA
gacgcgtgtctactcgaacata

SEQ ID NO: 9 - RNA, 22 nt, synthetic construct
  source 1..22: mol_type = other RNA
tgttcgagtagacacgcgtcac

SEQ ID NO: 10 - RNA, 22 nt, synthetic construct
  source 1..22: mol_type = other RNA
tgttcgagtagacacgcgtcac

SEQ ID NO: 11 - RNA, 500 nt, synthetic construct
  source 1..500: mol_type = other RNA
atgggggtggaactcatgatggaattggagcctttacaagggaatgaagagacaagagctctctttatgccacgtgaggatacagcaaggccccaatctgcaagccaggaagagtcgtcacgagaaccagaccatgcaggaactctgatcgtggacatttcaacctccagaactgtgatccaaaatgcatatgtatctttggaagaaactctgaagtaaaggccggaatattctttgtttaaaacattaaaaacaaaacagaccaaagcatcaagcaagaagtttcctggcaataaactaagcacagcattattttttaaggaacacaaattaagtgttcaacctgtggcaaatttgtactttctccctgaattatgttgttatcaaagaaaaaaattgggaagcatggcaaaatatcatcaaaactgaaactagaattaaacaaaactaaattaaaatgaaataaaatgatgtccattcttaaaaaaaaaaaaaaaaaa

SEQ ID NO: 12 - RNA, 3184 nt, synthetic construct
  source 1..3184: mol_type = other RNA
acatttgcttctgacacaactgtgttcactagcaacctcaaacagacaccatgggcgtgaagtccacactcgtgtccggctccaaagtgtacatgacaaccttcgccgaaggcagcgacgccaggctggaaaagatcgtggagggcgacagcatcaggagcgtgaatgagggcgaggccttcagcgctgaaatggccgataaaaacgccggctataagatcggcaacgccaaattcagccatcctaagggctacgccgtggtggctaacaaccctctgtatacaggacccgtccagcaggatatgctcggcctgaaggaaactctggaaaagaggtacttcggcgagagcgctgatggcaatgacaatatttgtatccaggtgatccataacatcctggacattgaaaaaatcctcgccgaatacattaccaacgccgcctacgccgtcaacaatatctccggcctggataaggacattattggattcggcaagttctccacagtgtatacctacgacgaattcaaagaccccgagcaccatagggccgctttcaacaataacgataagctcatcaacgccatcaaggcccagtatgacgagttcgacaacttcctcgataaccccagactcggctatttcggccaggcctttttcagcaaggagggcagaaattacatcatcaattacggcaacgaatgctatgacattctggccctcctgagcggactggcgcactgggtggtcgctaacaacgaagaagagtccaggatctccaggacctggctctacaacctcgataagaacctcgacaacgaatacatctccaccctcaactacctctacgacaggatcaccaatgagctgaccaactccttctccaagaactccgccgccaacgtgaactatattgccgaaactctgggaatcaaccctgccgaattcgccgaacaatatttcagattcagcattatgaaagagcagaaaaacctcggattcaatatcaccaagctcagggaagtgatgctggacaggaaggatatgtccgagatcaggaaaaatcataaggtgttcgactccatcaggaccaaggtctacaccatgatggactttgtgatttataggtattacatcgaagaggatgccaaggtggctgccgccaataagtccctccccgataatgagaagtccctgagcgagaaggatatctttgtgattaacctgaggggctccttcaacgacgaccagaaggatgccctctactacgatgaagctaatagaatttggagaaagctcgaaaatatcatgcacaacatcaaggaatttaggggaaacaagacaagagagtataagaagaaggacgcccctagactgcccagaatcctgcccgctggccgtgatgtttccgccttcagcaaactcatgtatgccctgaccatgttcctggatggcaaggagatcaacgacctcctgaccaccctgattaataaattcgataacatccagagcttcctgaaggtgatgcctctcatcggagtcaacgctaagttcgtggaggaatacgcctttttcaaagactccgccaagatcgccgatgagctgaggctgatcaagtccttcgctagaatgggagaacctattgccgatgccaggagggccatgtatatcgacgccatccgtattttaggaaccaacctgtcctatgatgagctcaaggccctcgccgacaccttttccctggacgagaacggaaacaagctcaagaaaggcaagcacggcatgagaaatttcattattaataacgtgatcagcaataaaaggttccactacctgatcagatacggtgatcctgcccacctccatgagatcgccaaaaacgaggccgtggtgaagttcgtgctcggcaggatcgctgacatccagaaaaaacagggccagaacggcaagaaccagatcgacaggtactacgaaacttgtatcggaaaggataagggcaagagcgtgagcgaaaaggtggacgctctcacaaagatcatcaccggaatgaactacgaccaattcgacaagaaaaggagcgtcattgaggacaccggcagggaaaacgccgagagggagaagtttaaaaagatcatcagcctgtacctcaccgtgatctaccacatcctcaagaatattgtcaatatcaacgccaggtacgtcatcggattccattgcgtcgagcgtgatgctcaactgtacaaggagaaaggctacgacatcaatctcaagaaactggaagagaagggattcagctccgtcaccaagctctgcgctggcattgatgaaactgcccccgataagagaaaggacgtggaaaaggagatggctgaaagagccaaggagagcattgacagcctcgagagcgccaaccccaagctgtatgccaattacatcaaatacagcgacgagaagaaagccgaggagttcaccaggcagattaacagggagaaggccaaaaccgccctgaacgcctacctgaggaacaccaagtggaatgtgatcatcagggaggacctcctgagaattgacaacaagacatgtaccctgttcgcaaacaaggccgtcgccctggaagtggccaggtatgtccacgcctatatcaacgacattgccgaggtcaattcctacttccaactgtaccattacatcatgcagagaattatcatgaatgagaggtacgagaaaagcagcggaaaggtgtccgagtacttcgacgctgtgaatgacgagaagaagtacaacgataggctcctgaaactgctgtgtgtgcctttcggctactgtatccccaggtttaagaacctgagcatcgaggccctgttcgataggaacgaggccgccaagttcgacaaggagaaaaagaaggtgtccggcaattccaccgtggaacggatcattcaggccctgcctccacttgaaagactgacactgtaagctcgctttcttgctgtccaatttctattaaaggttcctttgttccctaagtccaactactaaactgggggatattatgaagggccttgagcatctggattctgcctaataaaaaacatttattttcattgcaaaaaaaaaaaaaaaaaaaaaaaaaaaaaaaaaaaaaaaaaaaaaaaaaaaaaaaaaaaaaaaaaaaaaaaaaaaaaaaa

SEQ ID NO: 13 - RNA, 705 nt, synthetic construct
  source 1..705: mol_type = other RNA
ggtcccaggtccacttcaagtaaacccctaccaactggtcggggtttgaaacccaattccatcatgagttccaccgcgtgtggcctcgaacaccgagcgaccctgcagcgacccgcttaaaagcttggcaatccggtactgttggtaaagccaccatggtcttcacactcgaagatttcgttggggactggcgacagacagccggctacaacctggaccaagtccttgaacagggaggtgtgtccagtttgtttcagaatctcggggtgtccgtaactccgatccaaaggattgtcctgagcggtgaaaatgggctgaagatcgacatccatgtcatcatcccgtatgaaggtctgagcggcgaccaaatgggccagatcgaaaaaatttttaaggtggtgtaccctgtggatgatcatcactttaaggtgatcctgcactatggcacactggtaatcgacggggttacgccgaacatgatcgactatttcggacggccgtatgaaggcatcgccgtgttcgacggcaaaaagatcactgtaacagggaccctgtggaacggcaacaaaattatcgacgagcgcctgatcaaccccgacggctccctgctgttccgagtaaccatcaacggagtgaccggctggcggctgtgcgaacgcattctggcgtaattctaaaaaaaaaaaaaaaaaaaaaaaaaaaaaa

SEQ ID NO: 14 - RNA, 705 nt, synthetic construct
  source 1..705: mol_type = other RNA
ggtcccaggtccacttcaagtaaacccctaccaactggtcggggtttgaaacaggctccaattccatcatgagttgcgtgtggcctcgaacaccgagcgaccctgcagcgacccgcttaaaagcttggcaatccggtactgttggtaaagccaccatggtcttcacactcgaagatttcgttggggactggcgacagacagccggctacaacctggaccaagtccttgaacagggaggtgtgtccagtttgtttcagaatctcggggtgtccgtaactccgatccaaaggattgtcctgagcggtgaaaatgggctgaagatcgacatccatgtcatcatcccgtatgaaggtctgagcggcgaccaaatgggccagatcgaaaaaatttttaaggtggtgtaccctgtggatgatcatcactttaaggtgatcctgcactatggcacactggtaatcgacggggttacgccgaacatgatcgactatttcggacggccgtatgaaggcatcgccgtgttcgacggcaaaaagatcactgtaacagggaccctgtggaacggcaacaaaattatcgacgagcgcctgatcaaccccgacggctccctgctgttccgagtaaccatcaacggagtgaccggctggcggctgtgcgaacgcattctggcgtaattctaaaaaaaaaaaaaaaaaaaaaaaaaaaaaa

SEQ ID NO: 15 - RNA, 705 nt, synthetic construct
  source 1..705: mol_type = other RNA
ggtcccaggtccacttcaagtaaacccctaccaactggtcggggtttgaaactgtaaaggctccaattccatcatgcgtgtggcctcgaacaccgagcgaccctgcagcgacccgcttaaaagcttggcaatccggtactgttggtaaagccaccatggtcttcacactcgaagatttcgttggggactggcgacagacagccggctacaacctggaccaagtccttgaacagggaggtgtgtccagtttgtttcagaatctcggggtgtccgtaactccgatccaaaggattgtcctgagcggtgaaaatgggctgaagatcgacatccatgtcatcatcccgtatgaaggtctgagcggcgaccaaatgggccagatcgaaaaaatttttaaggtggtgtaccctgtggatgatcatcactttaaggtgatcctgcactatggcacactggtaatcgacggggttacgccgaacatgatcgactatttcggacggccgtatgaaggcatcgccgtgttcgacggcaaaaagatcactgtaacagggaccctgtggaacggcaacaaaattatcgacgagcgcctgatcaaccccgacggctccctgctgttccgagtaaccatcaacggagtgaccggctggcggctgtgcgaacgcattctggcgtaattctaaaaaaaaaaaaaaaaaaaaaaaaaaaaaa

SEQ ID NO: 16 - DNA, 30 bp, synthetic construct
  source 1..30: mol_type = other DNA
agtggacctgggaccttttttttttttttt

SEQ ID NO: 17 - RNA, 24 nt, synthetic construct
  source 1..24: mol_type = other RNA
aaaaggcgcatattaaggtgacgc

SEQ ID NO: 18 - RNA, 51 nt, synthetic construct
  source 1..51: mol_type = other RNA
gcgtcanccttaatatgcgccaaaaaaaaaaaaaaaaaaaaaaaaaaaaaa

SEQ ID NO: 19 - RNA, 51 nt, synthetic construct
  source 1..51: mol_type = other RNA
gcgtcaccttaatantgcgccaaaaaaaaaaaaaaaaaaaaaaaaaaaaaa

SEQ ID NO: 20 - RNA, 51 nt, synthetic construct; identical to SEQ ID NO: 19
  source 1..51: mol_type = other RNA

SEQ ID NO: 21 - RNA, 50 nt, synthetic construct
  source 1..50: mol_type = other RNA
gcgtcaccttaatatgcgccaaaaaaaaaaaaaaaaaaaaaaaaaaaaaa

SEQ ID NO: 22 - RNA, 650 nt, synthetic construct
  source 1..650: mol_type = other RNA
ggcgcatattaaggtgacgcgtgtggcctcgaacaccgagcgaccctgcagcgacccgcttaaaagcttggcaatccggtactgttggtaaagccaccatggtcttcacactcgaagatttcgttggggactggcgacagacagccggctacaacctggaccaagtccttgaacagggaggtgtgtccagtttgtttcagaatctcggggtgtccgtaactccgatccaaaggattgtcctgagcggtgaaaatgggctgaagatcgacatccatgtcatcatcccgtatgaaggtctgagcggcgaccaaatgggccagatcgaaaaaatttttaaggtggtgtaccctgtggatgatcatcactttaaggtgatcctgcactatggcacactggtaatcgacggggttacgccgaacatgatcgactatttcggacggccgtatgaaggcatcgccgtgttcgacggcaaaaagatcactgtaacagggaccctgtggaacggcaacaaaattatcgacgagcgcctgatcaaccccgacggctccctgctgttccgagtaaccatcaacggagtgaccggctggcggctgtgcgaacgcattctggcgtaattctagaaaaaaaaaaaaaaaaaaaaaaaaaaaaaa

SEQ ID NO: 23 - DNA, 30 bp, synthetic construct
  source 1..30: mol_type = other DNA
accttaatatgcgccttttttttttttttt

SEQ ID NO: 24 - DNA, 48 bp, synthetic construct
  source 1..48: mol_type = other DNA
cccggatcctaatacgactcactataggcgcatattaaggtgacgcgt

SEQ ID NO: 25 - DNA, 49 bp, synthetic construct
  source 1..49: mol_type = other DNA
cccggatcctaatacgactcactataaggcgcatattaaggtgacgcgt

SEQ ID NO: 26 - DNA, 49 bp, synthetic construct
  source 1..49: mol_type = other DNA
cccggatcctaatacgactcactatatggcgcatattaaggtgacgcgt

SEQ ID NO: 27 - DNA, 49 bp, synthetic construct
  source 1..49: mol_type = other DNA
cccggatcctaatacgactcactatacggcgcatattaaggtgacgcgt

SEQ ID NO: 28 - DNA, 49 bp, synthetic construct
  source 1..49: mol_type = other DNA
cccggatcctaatacgactcactatagggcgcatattaaggtgacgcgt

SEQ ID NO: 29 - DNA, 50 bp, synthetic construct
  source 1..50: mol_type = other DNA
cccggatcctaatacgactcactatatcggcgcatattaaggtgacgcgt

SEQ ID NO: 30 - DNA, 50 bp, synthetic construct
  source 1..50: mol_type = other DNA
cccggatcctaatacgactcactatataggcgcatattaaggtgacgcgt

SEQ ID NO: 31 - DNA, 50 bp, synthetic construct
  source 1..50: mol_type = other DNA
cccggatcctaatacgactcactatattggcgcatattaaggtgacgcgt

SEQ ID NO: 32 - DNA, 50 bp, synthetic construct
  source 1..50: mol_type = other DNA
cccggatcctaatacgactcactataccggcgcatattaaggtgacgcgt

SEQ ID NO: 33 - DNA, 50 bp, synthetic construct
  source 1..50: mol_type = other DNA
cccggatcctaatacgactcactatactggcgcatattaaggtgacgcgt

SEQ ID NO: 34 - DNA, 50 bp, synthetic construct
  source 1..50: mol_type = other DNA
cccggatcctaatacgactcactatacaggcgcatattaaggtgacgcgt

SEQ ID NO: 35 - DNA, 50 bp, synthetic construct
  source 1..50: mol_type = other DNA
cccggatcctaatacgactcactatagtggcgcatattaaggtgacgcgt

SEQ ID NO: 36 - DNA, 50 bp, synthetic construct
  source 1..50: mol_type = other DNA
cccggatcctaatacgactcactatagcggcgcatattaaggtgacgcgt

SEQ ID NO: 37 - DNA, 50 bp, synthetic construct
  source 1..50: mol_type = other DNA
cccggatcctaatacgactcactatagaggcgcatattaaggtgacgcgt

SEQ ID NO: 38 - DNA, 50 bp, synthetic construct
  source 1..50: mol_type = other DNA
cccggatcctaatacgactcactataatggcgcatattaaggtgacgcgt

SEQ ID NO: 39 - DNA, 50 bp, synthetic construct
  source 1..50: mol_type = other DNA
cccggatcctaatacgactcactataacggcgcatattaaggtgacgcgt

SEQ ID NO: 40 - DNA, 50 bp, synthetic construct
  source 1..50: mol_type = other DNA
cccggatcctaatacgactcactataaaggcgcatattaaggtgacgcgt

SEQ ID NO: 41 - DNA, 49 bp, synthetic construct
  source 1..49: mol_type = other DNA
cccggatcctaatacgactcactattaggcgcatattaaggtgacgcgt

SEQ ID NO: 42 - DNA, 50 bp, synthetic construct
  source 1..50: mol_type = other DNA
cccggatcctaatacgactcactatttaggcgcatattaaggtgacgcgt

SEQ ID NO: 43 - DNA, 50 bp, synthetic construct
  source 1..50: mol_type = other DNA
cccggatcctaatacgactcactatctaggcgcatattaaggtgacgcgt

SEQ ID NO: 44 - DNA, 50 bp, synthetic construct
  source 1..50: mol_type = other DNA
cccggatcctaatacgactcactatgtaggcgcatattaaggtgacgcgt

SEQ ID NO: 45 - DNA, 51 bp, synthetic construct
  source 1..51: mol_type = other DNA
ttttttttttttttttttttttttttttttctagaattacgccagaatgcg

SEQ ID NO: 46 - RNA, 87 nt, synthetic construct
  source 1..87: mol_type = other RNA
agagccaccatggtgagcggctggcggctgttcaagaagattagcgggagctccggtagtataatcaactttgaaaaactgtgataa

SEQ ID NO: 47 - RNA, 30 nt, synthetic construct
  source 1..30: mol_type = other RNA
aaaaaaaaaaaaaaaaaaaaaaaaaaaaaa

SEQ ID NO: 48 - RNA, 10 nt, synthetic construct
  source 1..10: mol_type = other RNA
ctcctagtcc

SEQ ID NO: 49 - RNA, 70 nt, synthetic construct
  source 1..70: mol_type = other RNA
gctggagcctcggtggccatgcttcttgccccttgggcctaaaaaaaaaaaaaaaaaaaaaaaaaaaaaa

SEQ ID NO: 50 - RNA, 10 nt, synthetic construct
  source 1..10: mol_type = other RNA
ctcctagtcc

SEQ ID NO: 51 - protein, 24 aa, synthetic construct
MVSGWRLFKKISGSSGSIINFEKL

SEQ ID NO: 52 - DNA, 25 bp, synthetic construct
  source 1..25: mol_type = other DNA
caccatggtggctctggactaggag

SEQ ID NO: 53 - DNA, 30 bp, synthetic construct
  source 1..30: mol_type = other DNA
tttttttttttttttttatcacagtttttc

SEQ ID NO: 54 - DNA, 30 bp, synthetic construct
  source 1..30: mol_type = other DNA
caccgaggctccagcttatcacagtttttc

SEQ ID NO: 55 - DNA, 25 bp, synthetic construct
  source 1..25: mol_type = other DNA
caccatggtggctctggactaggag

SEQ ID NO: 56 - RNA, 1679 nt, synthetic construct
  source 1..1679: mol_type = other RNA
gtgacattcttctggacaatgagtcccatcatctctccaccatgcaccttgtgactccctcctctgctgacaacagataaccacctttaactgtaactttccacagcctaccccagccctataaagctgcccctctcctatctcccttcgctgactctcttttcagactcagcccacttgcacccaagtgaattaacagccttgttgctcacacaaagcctgtttaggtggtcttctatacggacatgcttgacacttggtgccaaaatctgggccagggggactccttcgtgagaccggccccctgtcctggccctcattccgtgaagagatccacctgcgacctcgggtcctcagaccagcccaaggaacatctcaccaatttcaaatcggatctcctcggcttagtggctgaagactgatgctgcccgatcgcctcagaagccccttggaccatcacagatgccgagcttcgggtaactcttacggtggagggatctgcaatcagaactattgaacttctccattcagaccgccactcacacctatgggaaaagggtaatgtatcatcggcttagcaacagggaatactattcgtatgatggaaaatggggacaaaaggctttggtacataaaacattattccttccttggcctaaaaactcatcgccacctacattaaagctaatatgcctgattactgtttttagagaacttattttattagggcagttccaagctcaaaaatacgctaactggcaccttgttagctacataaaaatgcaccctagacccgaaacttactagactcattataaaattttctttaaggtgtccacgcagtccctggtcacacttgaagcagtccggagaaatatcagccctaccccagtaatccccagaaggaacttacacttttttttaatcttttcctacaacttcatattttataaataaaaagacaaaaatgtcaggcctgtgagctgaagcttagccattgtaacccctgtgacctgcacatatccgtccaggtggcctgcaggagccaagaagtctggagcagccgaaaaaccacaaagaagtgaaacagccagttcctgccttaactaattaacccaccttacgacattccaccattatgacttgtccaccattatgacttgttcctgccctgccccaactgatcaatcaaccctgtgacattcttctcctggacaatgagtcccatcatctctccaccatgcaccttgtgaccccctcctctgctgaggataaccacctttaactgtaactttccacgcctacccaagccctataaagctgcccctctcctatctcccttcactgactctcttttcggactcagcccacttgcacccaagtgaattaacagccttgttgctcacacaaagcctgattgggtgtcttctatacggacacgcgtgacaggaacctcaacccaaaggcagtctgatgaggtgtctaagataaaagtagcggcacaaaggcttttgtaaacagaggcgtttcatgtggttttcctttcctttccttatatgtgaaaaggtgacagaaaagaaatcttcctaaaagagtcagccactgctctgtggaacgatgatcatttaaatgccacgtcgatttgaaacgtacaacaaagggactaacagttgagaacc

SEQ ID NO: 57 - RNA, 705 nt, synthetic construct
  source 1..705: mol_type = other RNA
ggtcccaggtccacttcaagtaaacccctaccaactggtcggggtttgaaactggagagatgatgggactcattggcgtgtggcctcgaacaccgagcgaccctgcagcgacccgcttaaaagcttggcaatccggtactgttggtaaagccaccatggtcttcacactcgaagatttcgttggggactggcgacagacagccggctacaacctggaccaagtccttgaacagggaggtgtgtccagtttgtttcagaatctcggggtgtccgtaactccgatccaaaggattgtcctgagcggtgaaaatgggctgaagatcgacatccatgtcatcatcccgtatgaaggtctgagcggcgaccaaatgggccagatcgaaaaaatttttaaggtggtgtaccctgtggatgatcatcactttaaggtgatcctgcactatggcacactggtaatcgacggggttacgccgaacatgatcgactatttcggacggccgtatgaaggcatcgccgtgttcgacggcaaaaagatcactgtaacagggaccctgtggaacggcaacaaaattatcgacgagcgcctgatcaaccccgacggctccctgctgttccgagtaaccatcaacggagtgaccggctggcggctgtgcgaacgcattctggcgtaattctaaaaaaaaaaaaaaaaaaaaaaaaaaaaaa

SEQ ID NO: 58 - RNA, 201 nt, synthetic construct
  source 1..201: mol_type = other RNA
ggcgcatattaaggtgacgcgtgtggcctcgaacaccgagggtanaagccaccatggtgagcggctggcggctgttcaagaagattagcgggagctccggtagtataatcaactttgaaaaactgtgataagctggagcctcggtggccatgcttcttgccccttgggcctaaaaaaaaaaaaaaaaaaaaaaaaaaaaaa

SEQ ID NO: 59 - protein, 24 aa, synthetic construct
MVSGWRLFKKISGSSGSIINFEKL

SEQ ID NO: 60 - RNA, 23 nt, synthetic construct
  source 1..23: mol_type = other RNA
tacctgtacactgacttgagatt

SEQ ID NO: 61 - RNA, 23 nt, synthetic construct
  source 1..23: mol_type = other RNA
tctcaagtcagtgtacaggtatt

SEQ ID NO: 62 - RNA, 682 nt, synthetic construct
  source 1..682: mol_type = other RNA
ggtcccaggtccacttcaagtaaacccctaccaactggtcggggtttgaaacgcgtgtggcctcgaacaccgagcgaccctgcagcgacccgcttaaaagcttggcaatccggtactgttggtaaagccaccatggtcttcacactcgaagatttcgttggggactggcgacagacagccggctacaacctggaccaagtccttgaacagggaggtgtgtccagtttgtttcagaatctcggggtgtccgtaactccgatccaaaggattgtcctgagcggtgaaaatgggctgaagatcgacatccatgtcatcatcccgtatgaaggtctgagcggcgaccaaatgggccagatcgaaaaaatttttaaggtggtgtaccctgtggatgatcatcactttaaggtgatcctgcactatggcacactggtaatcgacggggttacgccgaacatgatcgactatttcggacggccgtatgaaggcatcgccgtgttcgacggcaaaaagatcactgtaacagggaccctgtggaacggcaacaaaattatcgacgagcgcctgatcaaccccgacggctccctgctgttccgagtaaccatcaacggagtgaccggctggcggctgtgcgaacgcattctggcgtaattctaaaaaaaaaaaaaaaaaaaaaaaaaaaaaa

SEQ ID NO: 63 - RNA, 705 nt, synthetic construct
  source 1..705: mol_type = other RNA
ggtcccaggtccacttcaagtaaacccctaccaactggtcggggtttgaaacggcaaaggcgaggctctgtgctcgcgtgtggcctcgaacaccgagcgaccctgcagcgacccgcttaaaagcttggcaatccggtactgttggtaaagccaccatggtcttcacactcgaagatttcgttggggactggcgacagacagccggctacaacctggaccaagtccttgaacagggaggtgtgtccagtttgtttcagaatctcggggtgtccgtaactccgatccaaaggattgtcctgagcggtgaaaatgggctgaagatcgacatccatgtcatcatcccgtatgaaggtctgagcggcgaccaaatgggccagatcgaaaaaatttttaaggtggtgtaccctgtggatgatcatcactttaaggtgatcctgcactatggcacactggtaatcgacggggttacgccgaacatgatcgactatttcggacggccgtatgaaggcatcgccgtgttcgacggcaaaaagatcactgtaacagggaccctgtggaacggcaacaaaattatcgacgagcgcctgatcaaccccgacggctccctgctgttccgagtaaccatcaacggagtgaccggctggcggctgtgcgaacgcattctggcgtaattctaaaaaaaaaaaaaaaaaaaaaaaaaaaaaa

SEQ ID NO: 64 - RNA, 24 nt, synthetic construct
  source 1..24: mol_type = other RNA
gaggccacacgcgtttcaaacccc

SEQ ID NO: 65 - RNA, 24 nt, synthetic construct
  source 1..24: mol_type = other RNA
ctcgcctttgccgtttcaaacccc

SEQ ID NO: 66 - RNA, 24 nt, synthetic construct
  source 1..24: mol_type = other RNA
gaggccacacgcgagcacagagcc

SEQ ID NO: 67 - RNA, 682 nt, synthetic construct
  source 1..682: mol_type = other RNA
gcgtgtggcctcgaacaccgagcgaccctgcagcgacccgcttaaaagcttggcaatccggtactgttggtaaagccaccatggtcttcacactcgaagatttcgttggggactggcgacagacagccggctacaacctggaccaagtccttgaacagggaggtgtgtccagtttgtttcagaatctcggggtgtccgtaactccgatccaaaggattgtcctgagcggtgaaaatgggctgaagatcgacatccatgtcatcatcccgtatgaaggtctgagcggcgaccaaatgggccagatcgaaaaaatttttaaggtggtgtaccctgtggatgatcatcactttaaggtgatcctgcactatggcacactggtaatcgacggggttacgccgaacatgatcgactatttcggacggccgtatgaaggcatcgccgtgttcgacggcaaaaagatcactgtaacagggaccctgtggaacggcaacaaaattatcgacgagcgcctgatcaaccccgacggctccctgctgttccgagtaaccatcaacggagtgaccggctggcggctgtgcgaacgcattctggcgtaattctaaaaaaaaaaaaaaaaaaaaaaaaaaaaaaggtcccaggtccacttcaagtaaacccctaccaactggtcggggtttgaaac

SEQ ID NO: 68 - RNA, 47 nt, synthetic construct
  source 1..47: mol_type = other RNA
ggggtttgaaacggcaaaggcgaggctctgtgctcgcgtgtggcctc

SEQ ID NO: 69 - RNA, 200 nt, synthetic construct
  source 1..200: mol_type = other RNA
  modified_base 1..200: mod_base = m1f
ggcgcatattaaggtgacgcgtgtggcctcgaacaccgagggtaaagccaccatggngagcggcnggcggcngnncaagaagannagcgggagcnccggnagnanaancaacnnngaaaaacngnganaagcnggagccncggnggccangcnncnngccccnngggccnaaaaaaaaaaaaaaaaaaaaaaaaaaaaaa

SEQ ID NO: 70 - RNA, 816 nt, synthetic construct
  source 1..816: mol_type = other RNA
ggttaaaacagcggatgggtaccccaccatccgacccactgggtgtagtactctggtacttcgtacctttgtacgcctgttcttcccattgtacccttcctgaacttccaacccaagtaacgttagaagctcaacatttagtacaacaggaagcaccacatccagtggtgtttagtacaagcacttctgtttccccggagcgaggtataggctgtacccactgccaaaaacctttaaccgttatccgccaaccaactacgtaaaagctagtagtattatgtttttaactaggcgttcgatcaggtggatttcccctccactagtttggtcgatgaggctaggaattccccacgggtgaccgtgtcctagcctgcgtggcggccaacccagcccactcactatttgttttcgcgcccagttgcaaaaagtgtcggggctgggacgcctttttatagacatggtgtgaagactcgcatgtgcttggttgtgattcctccggcccctgaatgcggctaaccttaaccctggagccttgtgtcacaaaccagtgatgataaggtcgtaatgagcaattccgggacgggaccgactactttgggtgtccgtgtttcttatttttcttattattgtcttatggtcacagcatatatataacatatactgtgatcatggtgagcggctggcggctgttcaagaagattagcgggagctccggtagtataatcaactttgaaaaactgtgataagctggagcctcggtggccatgcttcttgccccttgggcctaaaaaaaaaaaaaaaaaaaaaaaaaaaaaa

SEQ ID NO: 71 - RNA, 816 nt, synthetic construct
  source 1..816: mol_type = other RNA
  modified_base 1..816: mod_base = m1f
ggnnaaaacagcggangggnaccccaccanccgacccacngggngnagnacncnggnacnncgnaccnnngnacgccngnncnncccanngnacccnnccngaacnnccaacccaagnaacgnnagaagcncaacannnagnacaacaggaagcaccacanccagnggngnnnagnacaagcacnncngnnnccccggagcgaggnanaggcngnacccacngccaaaaaccnnnaaccgnnanccgccaaccaacnacgnaaaagcnagnagnannangnnnnnaacnaggcgnncgancaggnggannnccccnccacnagnnnggncgangaggcnaggaannccccacgggngaccgngnccnagccngcgnggcggccaacccagcccacncacnannngnnnncgcgcccagnngcaaaaagngncggggcngggacgccnnnnnanagacanggngngaagacncgcangngcnnggnngngannccnccggccccngaangcggcnaaccnnaacccnggagccnngngncacaaaccagnganganaaggncgnaangagcaannccgggacgggaccgacnacnnngggngnccgngnnncnnannnnncnnannanngncnnanggncacagcananananaacananacngngancanggngagcggcnggcggcngnncaagaagannagcgggagcnccggnagnanaancaacnnngaaaaacngnganaagcnggagccncggnggccangcnncnngccccnngggccnaaaaaaaaaaaaaaaaaaaaaaaaaaaaaa